European Patent Application EP 4 810 514 A1, published September 23, 2026. Title: SKP2 FRAGMENT AND VARIANTS THEREOF, AND USE THEREOF. Applicant: 주식회사 제넥신. The sequence listing filed with the application follows.

SEQUENCE LISTING (66 sequences)

SEQ ID NO: 1 - protein, 175 aa, synthetic construct
  REGION 1..175: note = SKP2 fragment(2-176)
HRKHLQEIPDLSSNVATSFTWGWDSSKTSELLSGMGVSALEKEEPDSENIPQELLSNLGHPESPPRKRLKSKGSDKDFVIVRRPKLNRENFPGVSWDSLPDELLLGIFSCLCLPELLKVSGVCKRWYRLASDESLWQTLDLTGKNLHPDVTGRLLSQGVIAFRCPRSFMDQPLAE

SEQ ID NO: 2 - protein, 175 aa, synthetic construct
  REGION 1..175: note = variant 3 of SKP2 fragment(2-176)
RRRHLQEIPGLSSNVATSFTWGRDSSKTSELLSGMGVSALEKEEPDSENIPQELLSNPGHPESPPRKRLKSKGSDKDFVIVRRPKLNRENFPGVSWDSLPDELLLRIFSRLRLPELLKVSGVCKRWYRLASDESLWKTLDLTGKNLHPDVTGRLLSQGVVAFRCPRSFMDQPLAG

SEQ ID NO: 3 - protein, 175 aa, synthetic construct
  REGION 1..175: note = variant 15 of SKP2 fragment(2-176)
HRKHLQEIPDPSSNVATSFTWGWDSSKTSELPSGMGVSALEKEEPDSENIPQELLSNLGHPESPPRKRLKSKGSDKGFVIVRRPKLNRENFPGVSWVSLPDELLLGIFSCLCLPELLKVSGVCKRWCRLASDEPLWQTLDLTGKNLRPDVTGRLLSQGVIAFRCPRSFMDQPLAE

SEQ ID NO: 4 - protein, 175 aa, synthetic construct
  REGION 1..175: note = E1 variant
RRRHLQEIPGLSSNVATSFTWGRDSSKTSELLSGMGVSALEKEEPDSENIPQELLSNPGHPESPPRKRLKSKGSDKDFVIVRRPKLNRENFPGVSWDSLPDELLLRIFSRLRLPELLKVSGVSKRWYRLASDESLWKSLDLTGKNLHPDVTGRLLSQGVVAFRCPRSFMDQPLAG

SEQ ID NO: 5 - protein, 175 aa, synthetic construct
  REGION 1..175: note = E2 variant
RRRHLQEIPGLSSNVATSFTWGRDSSKTSELLSGMGVSALEKEEPDSENIPQELLSNPGHPESPPRKRLKSKGSDKDFVIVRRPKLNRENFPGVSWDSLPDELLLRIFSRLRLPELLKVSGVSKRWCRLASDESLWKTLDLTGKNLHPDVTGRLLSQGVAAFRCPRSFMDQPLAG

SEQ ID NO: 6 - protein, 175 aa, synthetic construct
  REGION 1..175: note = E4 variant
HRKHLQEIPDPSSNVATSFTWGWDSSKTSELPSGMGVSALEKEEPDSENIPQELLSNLGHPESPPRKRLKSKGSDKGFVIVRRPKLNRENFPGVSWVSLPDELLLGIFSCPCLPELLKVSGVCKRWCRLASDEPLWQTLDLTGKNLRPDVTGRLRSQGVIAFRCPRSFMDQPLAE

SEQ ID NO: 7 - protein, 175 aa, synthetic construct
  REGION 1..175: note = E5 variant
HRKHLQEIPDPSSNVATSFTWGWDSSKTSELPSGMGVSALEKKEPDSENIPQELLSNLGHPESPPRKRLKSKGSDKGFVIVRRPKLNRENFPGVSWVSLPDELLLGIFSCPCLPELLKVSGVCKRWCRLASDEPLRQTLDLTGKNLRPDVTGRLLSQGVIAFRCPRSFMDQPLAE

SEQ ID NO: 8 - protein, 175 aa, synthetic construct
  REGION 1..175: note = E6 variant
HRKHLQEIPDPSSNVATGFTWGWDSSKASELPSGMGVSALEKEEPDSENIPQELLSNLGHPESPPRKRLKSKGSDKGFVIVRRPKLNRENFPGVSWVSLPNELLLGIFSCRCLPELLKVSGVCKRWCRQASEEPLWQTLDLTGKNLRPDVTGRLQSQGVIAFRCPRSFMDQPLAE

SEQ ID NO: 9 - protein, 309 aa, synthetic construct
  REGION 1..309: note = Flag tag-SKP2(2-176).GS.NbALFA
DYKDDDDKTRHRKHLQEIPDLSSNVATSFTWGWDSSKTSELLSGMGVSALEKEEPDSENIPQELLSNLGHPESPPRKRLKSKGSDKDFVIVRRPKLNRENFPGVSWDSLPDELLLGIFSCLCLPELLKVSGVCKRWYRLASDESLWQTLDLTGKNLHPDVTGRLLSQGVIAFRCPRSFMDQPLAEGSEVQLQESGGGLVQPGGSLRLSCTASGVTISALNAMAMGWYRQAPGERRVMVAAVSERGNAMYRESVQGRFTVTRDFTNKMVSLQMDNLKPEDTAVYYCHVLEDRVDSFHDYWGQGTQVTVSS

SEQ ID NO: 10 - protein, 309 aa, synthetic construct
  REGION 1..309: note = Flag tag-E1.GS.NbALFA
DYKDDDDKTRRRRHLQEIPGLSSNVATSFTWGRDSSKTSELLSGMGVSALEKEEPDSENIPQELLSNPGHPESPPRKRLKSKGSDKDFVIVRRPKLNRENFPGVSWDSLPDELLLRIFSRLRLPELLKVSGVSKRWYRLASDESLWKSLDLTGKNLHPDVTGRLLSQGVVAFRCPRSFMDQPLAGGSEVQLQESGGGLVQPGGSLRLSCTASGVTISALNAMAMGWYRQAPGERRVMVAAVSERGNAMYRESVQGRFTVTRDFTNKMVSLQMDNLKPEDTAVYYCHVLEDRVDSFHDYWGQGTQVTVSS

SEQ ID NO: 11 - protein, 309 aa, synthetic construct
  REGION 1..309: note = Flag tag-E2.GS.NbALFA
DYKDDDDKTRRRRHLQEIPGLSSNVATSFTWGRDSSKTSELLSGMGVSALEKEEPDSENIPQELLSNPGHPESPPRKRLKSKGSDKDFVIVRRPKLNRENFPGVSWDSLPDELLLRIFSRLRLPELLKVSGVSKRWCRLASDESLWKTLDLTGKNLHPDVTGRLLSQGVAAFRCPRSFMDQPLAGGSEVQLQESGGGLVQPGGSLRLSCTASGVTISALNAMAMGWYRQAPGERRVMVAAVSERGNAMYRESVQGRFTVTRDFTNKMVSLQMDNLKPEDTAVYYCHVLEDRVDSFHDYWGQGTQVTVSS

SEQ ID NO: 12 - protein, 309 aa, synthetic construct
  REGION 1..309: note = Flag tag-E4.GS.NbALFA
DYKDDDDKTRHRKHLQEIPDPSSNVATSFTWGWDSSKTSELPSGMGVSALEKEEPDSENIPQELLSNLGHPESPPRKRLKSKGSDKGFVIVRRPKLNRENFPGVSWVSLPDELLLGIFSCPCLPELLKVSGVCKRWCRLASDEPLWQTLDLTGKNLRPDVTGRLRSQGVIAFRCPRSFMDQPLAEGSEVQLQESGGGLVQPGGSLRLSCTASGVTISALNAMAMGWYRQAPGERRVMVAAVSERGNAMYRESVQGRFTVTRDFTNKMVSLQMDNLKPEDTAVYYCHVLEDRVDSFHDYWGQGTQVTVSS

SEQ ID NO: 13 - protein, 309 aa, synthetic construct
  REGION 1..309: note = Flag tag-E5.GS.NbALFA
DYKDDDDKTRHRKHLQEIPDPSSNVATSFTWGWDSSKTSELPSGMGVSALEKKEPDSENIPQELLSNLGHPESPPRKRLKSKGSDKGFVIVRRPKLNRENFPGVSWVSLPDELLLGIFSCPCLPELLKVSGVCKRWCRLASDEPLRQTLDLTGKNLRPDVTGRLLSQGVIAFRCPRSFMDQPLAEGSEVQLQESGGGLVQPGGSLRLSCTASGVTISALNAMAMGWYRQAPGERRVMVAAVSERGNAMYRESVQGRFTVTRDFTNKMVSLQMDNLKPEDTAVYYCHVLEDRVDSFHDYWGQGTQVTVSS

SEQ ID NO: 14 - protein, 309 aa, synthetic construct
  REGION 1..309: note = Flag tag-E6.GS.NbALFA
DYKDDDDKTRHRKHLQEIPDPSSNVATGFTWGWDSSKASELPSGMGVSALEKEEPDSENIPQELLSNLGHPESPPRKRLKSKGSDKGFVIVRRPKLNRENFPGVSWVSLPNELLLGIFSCRCLPELLKVSGVCKRWCRQASEEPLWQTLDLTGKNLRPDVTGRLQSQGVIAFRCPRSFMDQPLAEGSEVQLQESGGGLVQPGGSLRLSCTASGVTISALNAMAMGWYRQAPGERRVMVAAVSERGNAMYRESVQGRFTVTRDFTNKMVSLQMDNLKPEDTAVYYCHVLEDRVDSFHDYWGQGTQVTVSS

SEQ ID NO: 15 - protein, 800 aa, synthetic construct
  REGION 1..800: note = ALFA-Myc tag.STAT3
SRLEEELRRRLTEPGSEQKLISEEDLGGGGSAQWNQLQQLDTRYLEQLHQLYSDSFPMELRQFLAPWIESQDWAYAASKESHATLVFHNLLGEIDQQYSRFLQESNVLYQHNLRRIKQFLQSRYLEKPMEIARIVARCLWEESRLLQTAATAAQQGGQANHPTAAVVTEKQQMLEQHLQDVRKRVQDLEQKMKVVENLQDDFDFNYKTLKSQGDMQDLNGNNQSVTRQKMQQLEQMLTALDQMRRSIVSELAGLLSAMEYVQKTLTDEELADWKRRQQIACIGGPPNICLDRLENWITSLAESQLQTRQQIKKLEELQQKVSYKGDPIVQHRPMLEERIVELFRNLMKSAFVVERQPCMPMHPDRPLVIKTGVQFTTKVRLLVKFPELNYQLKIKVCIDKDSGDVAALRGSRKFNILGTNTKVMNMEESNNGSLSAEFKHLTLREQRCGNGGRANCDASLIVTEELHLITFETEVYHQGLKIDLETHSLPVVVISNICQMPNAWASILWYNMLTNNPKNVNFFTKPPIGTWDQVAEVLSWQFSSTTKRGLSIEQLTTLAEKLLGPGVNYSGCQITWAKFCKENMAGKGFSFWVWLDNIIDLVKKYILALWNEGYIMGFISKERERAILSTKPPGTFLLRFSESSKEGGVTFTWVEKDISGKTQIQSVEPYTKQQLNNMSFAEIIMGYKIMDATNILVSPLVYLYPDIPKEEAFGKYCRPESQEHPEADPGSAAPYLKTKFICVTPTTCSNTIDLPMSPRTLDSLMQFGNNGEGAEPSAGGQFESLTFDMELTSECATSPM

SEQ ID NO: 16 - protein, 784 aa, synthetic construct
  REGION 1..784: note = Myc tag.STAT3
EQKLISEEDLGGGGSAQWNQLQQLDTRYLEQLHQLYSDSFPMELRQFLAPWIESQDWAYAASKESHATLVFHNLLGEIDQQYSRFLQESNVLYQHNLRRIKQFLQSRYLEKPMEIARIVARCLWEESRLLQTAATAAQQGGQANHPTAAVVTEKQQMLEQHLQDVRKRVQDLEQKMKVVENLQDDFDFNYKTLKSQGDMQDLNGNNQSVTRQKMQQLEQMLTALDQMRRSIVSELAGLLSAMEYVQKTLTDEELADWKRRQQIACIGGPPNICLDRLENWITSLAESQLQTRQQIKKLEELQQKVSYKGDPIVQHRPMLEERIVELFRNLMKSAFVVERQPCMPMHPDRPLVIKTGVQFTTKVRLLVKFPELNYQLKIKVCIDKDSGDVAALRGSRKFNILGTNTKVMNMEESNNGSLSAEFKHLTLREQRCGNGGRANCDASLIVTEELHLITFETEVYHQGLKIDLETHSLPVVVISNICQMPNAWASILWYNMLTNNPKNVNFFTKPPIGTWDQVAEVLSWQFSSTTKRGLSIEQLTTLAEKLLGPGVNYSGCQITWAKFCKENMAGKGFSFWVWLDNIIDLVKKYILALWNEGYIMGFISKERERAILSTKPPGTFLLRFSESSKEGGVTFTWVEKDISGKTQIQSVEPYTKQQLNNMSFAEIIMGYKIMDATNILVSPLVYLYPDIPKEEAFGKYCRPESQEHPEADPGSAAPYLKTKFICVTPTTCSNTIDLPMSPRTLDSLMQFGNNGEGAEPSAGGQFESLTFDMELTSECATSPM

SEQ ID NO: 17 - protein, 314 aa, synthetic construct
  REGION 1..314: note = Flag tag-SKP2(2-176).GS.ETI01_A4
DYKDDDDKTRHRKHLQEIPDLSSNVATSFTWGWDSSKTSELLSGMGVSALEKEEPDSENIPQELLSNLGHPESPPRKRLKSKGSDKDFVIVRRPKLNRENFPGVSWDSLPDELLLGIFSCLCLPELLKVSGVCKRWYRLASDESLWQTLDLTGKNLHPDVTGRLLSQGVIAFRCPRSFMDQPLAEGSHVQLVESGGGSVQAGGSLRLSCAASGFNSGDSCIGWFRQVPGKEREGVSVISSGGEIRYYADSVKGRFTISQDNTKNTLYLQMNSLKPEDTAMYYCATSVFLCYPRTWFNRYMYNSWGQGTQVTVSS

SEQ ID NO: 18 - protein, 314 aa, synthetic construct
  REGION 1..314: note = Flag tag-E1.GS.ETI01_A4
DYKDDDDKTRRRRHLQEIPGLSSNVATSFTWGRDSSKTSELLSGMGVSALEKEEPDSENIPQELLSNPGHPESPPRKRLKSKGSDKDFVIVRRPKLNRENFPGVSWDSLPDELLLRIFSRLRLPELLKVSGVSKRWYRLASDESLWKSLDLTGKNLHPDVTGRLLSQGVVAFRCPRSFMDQPLAGGSHVQLVESGGGSVQAGGSLRLSCAASGFNSGDSCIGWFRQVPGKEREGVSVISSGGEIRYYADSVKGRFTISQDNTKNTLYLQMNSLKPEDTAMYYCATSVFLCYPRTWFNRYMYNSWGQGTQVTVSS

SEQ ID NO: 19 - protein, 314 aa, synthetic construct
  REGION 1..314: note = Flag tag-E2.GS.ETI01_A4
DYKDDDDKTRRRRHLQEIPGLSSNVATSFTWGRDSSKTSELLSGMGVSALEKEEPDSENIPQELLSNPGHPESPPRKRLKSKGSDKDFVIVRRPKLNRENFPGVSWDSLPDELLLRIFSRLRLPELLKVSGVSKRWCRLASDESLWKTLDLTGKNLHPDVTGRLLSQGVAAFRCPRSFMDQPLAGGSHVQLVESGGGSVQAGGSLRLSCAASGFNSGDSCIGWFRQVPGKEREGVSVISSGGEIRYYADSVKGRFTISQDNTKNTLYLQMNSLKPEDTAMYYCATSVFLCYPRTWFNRYMYNSWGQGTQVTVSS

SEQ ID NO: 20 - protein, 314 aa, synthetic construct
  REGION 1..314: note = Flag tag-E4.GS.ETI01_A4
DYKDDDDKTRHRKHLQEIPDPSSNVATSFTWGWDSSKTSELPSGMGVSALEKEEPDSENIPQELLSNLGHPESPPRKRLKSKGSDKGFVIVRRPKLNRENFPGVSWVSLPDELLLGIFSCPCLPELLKVSGVCKRWCRLASDEPLWQTLDLTGKNLRPDVTGRLRSQGVIAFRCPRSFMDQPLAEGSHVQLVESGGGSVQAGGSLRLSCAASGFNSGDSCIGWFRQVPGKEREGVSVISSGGEIRYYADSVKGRFTISQDNTKNTLYLQMNSLKPEDTAMYYCATSVFLCYPRTWFNRYMYNSWGQGTQVTVSS

SEQ ID NO: 21 - protein, 314 aa, synthetic construct
  REGION 1..314: note = Flag tag-E5.GS.ETI01_A4
DYKDDDDKTRHRKHLQEIPDPSSNVATSFTWGWDSSKTSELPSGMGVSALEKKEPDSENIPQELLSNLGHPESPPRKRLKSKGSDKGFVIVRRPKLNRENFPGVSWVSLPDELLLGIFSCPCLPELLKVSGVCKRWCRLASDEPLRQTLDLTGKNLRPDVTGRLLSQGVIAFRCPRSFMDQPLAEGSHVQLVESGGGSVQAGGSLRLSCAASGFNSGDSCIGWFRQVPGKEREGVSVISSGGEIRYYADSVKGRFTISQDNTKNTLYLQMNSLKPEDTAMYYCATSVFLCYPRTWFNRYMYNSWGQGTQVTVSS

SEQ ID NO: 22 - protein, 7 aa, synthetic construct
  REGION 1..5: note = Flag tag-E6.GS.ETI01_A4
AAAAAAA

SEQ ID NO: 23 - DNA, 525 bp, synthetic construct
  source 1..525: mol_type = other DNA
  misc_feature 1..525: note = nucleotide sequence of SKP2 fragment(2-176)
cacaggaagcacctccaggagattccagacctgagtagcaacgttgccaccagcttcacgtggggatgggattccagcaagacttctgaactgctgtcaggcatgggggtctccgccctggagaaagaggagcccgacagtgagaacatcccccaggaactgctctcaaacctgggccacccggagagccccccacggaaacggctgaagagcaaagggagtgacaaagactttgtgattgtccgcaggcctaagctaaatcgagagaactttccaggtgtttcatgggactcccttccggatgagctgctcttgggaatcttttcctgtctgtgcctccctgagctgctaaaggtctctggtgtttgtaagaggtggtatcgcctagcgtctgatgagtctctatggcagaccttagacctcacaggtaaaaatctgcacccggatgtgactggtcggttgctgtctcaaggggtgattgccttccgctgcccacgatcatttatggaccaaccattggctgaa

SEQ ID NO: 24 - DNA, 15 bp, synthetic construct
  source 1..15: mol_type = other DNA
  misc_feature 1..15: note = nucleotide sequence of variant 3 of SKP2 fragment(2-176)
aaaaaaaaaaaaaaa

SEQ ID NO: 25 - DNA, 525 bp, synthetic construct
  source 1..525: mol_type = other DNA
  misc_feature 1..525: note = nucleotide sequence of variant 15 of SKP2 fragment(2-176)
cacaggaagcacctccaggagattccagacccgagtagcaacgttgccaccagcttcacgtggggatgggattccagcaagacttctgaactgccgtcaggcatgggggtctccgccctggagaaagaggagcccgacagtgagaatatcccccaggaactgctctcaaacctgggccacccggagagccccccacggaaacggctgaagagcaaagggagtgacaaaggctttgtgattgtccgcaggcctaagctaaatcgagagaactttccaggtgtttcgtgggtctcccttccggatgagctgctcttgggaatcttttcctgtctgtgcctccctgagctgctaaaggtctctggtgtttgcaagaggtggtgtcgcctagcgtctgatgagcctctatggcagaccttagacctcacaggtaaaaatctgcgcccggatgtgactggtcggttgctgtctcaaggggtgattgccttccgctgccctcgatcatttatggaccaaccattggccgaa

SEQ ID NO: 26 - DNA, 525 bp, synthetic construct
  source 1..525: mol_type = other DNA
  misc_feature 1..525: note = nucleotide sequence of E1 variant
cgcaggaggcacctccaggagattccaggcctgagtagcaacgttgccaccagcttcacgtggggacgggattccagcaagacttctgaactgctgtcaggcatgggggtctccgccctggagaaagaggagcccgacagtgagaacatcccccaggaactgctctcaaacccgggccacccggagagccccccacggaaacggctgaagagcaaagggagtgacaaagactttgtgattgtccgcaggcctaagctaaaccgagagaactttccaggcgtttcatgggactcccttccggatgagctgctcttgagaatcttttcccgtctgcgcctccctgagctgctaaaggtctctggtgttagtaagaggtggtatcgcctagcgtctgatgagtctctatggaagagcttagacctcacaggtaaaaatctgcacccggatgtgactggtcggttgctgtcccaaggggtggttgccttccgctgcccacgatcatttatggaccaaccattggctgga

SEQ ID NO: 27 - DNA, 525 bp, synthetic construct
  source 1..525: mol_type = other DNA
  misc_feature 1..525: note = nucleotide sequence of E2 variant
cgcaggaggcacctccaggagattccaggcctgagtagcaacgttgccaccagcttcacgtggggacgggattccagcaagacttctgaactgctgtcaggcatgggggtctccgccctggagaaagaggagcccgacagtgagaacatcccccaggaactgctctcaaacccgggccacccggagagccccccacggaaacggctgaagagcaaagggagtgacaaagactttgtgattgtccgcaggcctaagctaaaccgagagaactttccaggcgtttcatgggactcccttccggatgagctgctcttgagaatcttttcccgtctgcgcctccctgagctgctaaaggtctctggtgttagtaagaggtggtgtcgcctagcgtctgatgagtctctatggaagaccttagacctcacaggtaaaaatctgcacccggatgtgactggtcggttgctgtcccaaggggtggctgccttccgctgcccacgatcatttatggaccaaccattggctgga

SEQ ID NO: 28 - DNA, 525 bp, synthetic construct
  source 1..525: mol_type = other DNA
  misc_feature 1..525: note = nucleotide sequence of E4 variant
cacaggaagcacctccaggagattccagacccgagtagcaacgttgccaccagcttcacgtggggatgggattccagcaagacttctgaactgccgtcaggcatgggggtctccgccctggagaaagaggagcccgacagtgagaatatcccccaggaactgctctcaaacctgggccacccggagagccccccacggaaacggctgaagagcaaagggagtgacaaaggctttgtgattgtccgcaggcctaagctaaatcgagagaactttccaggtgtttcgtgggtctcccttccggatgagctgctcttgggaatcttttcctgtccgtgcctccctgagctgctaaaggtctctggtgtttgcaagaggtggtgtcgcctagcgtctgatgagcctctatggcagaccttagacctcacaggtaaaaatctgcgcccggatgtgactggtcggttgcggtctcaaggggtgattgccttccgctgccctcggtcatttatggaccaaccattggccgaa

SEQ ID NO: 29 - DNA, 525 bp, synthetic construct
  source 1..525: mol_type = other DNA
  misc_feature 1..525: note = nucleotide sequence of E5 variant
cacaggaagcacctccaggagattccagacccgagtagcaacgttgccaccagcttcacgtggggatgggattccagcaagacttctgaactgccgtcaggcatgggggtctccgccctggagaaaaaggagcccgacagtgagaatatcccccaggaactgctctcaaacctgggccacccggagagccccccacggaaacggctgaagagcaaagggagtgacaaaggctttgtgattgtccgcaggcctaagctaaatcgtgagaactttccaggtgtttcgtgggtctcccttccggatgagctgctcttgggaatcttttcctgtccgtgcctccctgagctgctaaaggtctctggtgtttgcaagaggtggtgtcgcctagcgtctgatgagcctctaaggcagaccttagacctcacaggtaaaaatctgcgcccggatgtgactggtcggttgctgtctcaaggggtgattgccttccgctgccctcgatcatttatggaccaaccattggccgaa

SEQ ID NO: 30 - DNA, 525 bp, synthetic construct
  source 1..525: mol_type = other DNA
  misc_feature 1..525: note = nucleotide sequence of E6 variant
cacaggaagcacctccaggagattccagacccgagtagcaacgttgccaccggcttcacgtggggatgggattccagcaaggcttctgaactgccgtcaggcatgggggtctccgccctggagaaagaggagcccgacagtgagaatatcccccaggaactgctctcaaacctgggccacccggagagccccccacggaaacggctgaagagcaaagggagtgacaaaggctttgtgattgtccgcaggcctaagctaaatcgagagaactttccaggtgtttcgtgggtctcccttccgaatgagctgctcttgggaatcttttcctgtcggtgcctccctgagctgctaaaggtctctggtgtttgtaagaggtggtgtcgccaagcgtctgaagagcctctatggcagaccttagacctcacaggtaaaaatctgcgcccggatgtgactggtcggttgcagtctcaaggggtgattgccttccgctgccctcgatcatttatggaccaaccattggctgaa

SEQ ID NO: 31 - DNA, 927 bp, synthetic construct
  source 1..927: mol_type = other DNA
  misc_feature 1..927: note = nucleotide sequence of Flag tag-SKP2(2-176).GS.NbALFA
gactacaaggacgacgatgacaagacgcgtcacaggaagcacctccaggagattccagacctgagtagcaacgttgccaccagcttcacgtggggatgggattccagcaagacttctgaactgctgtcaggcatgggggtctccgccctggagaaagaggagcccgacagtgagaacatcccccaggaactgctctcaaacctgggccacccggagagccccccacggaaacggctgaagagcaaagggagtgacaaagactttgtgattgtccgcaggcctaagctaaatcgagagaactttccaggtgtttcatgggactcccttccggatgagctgctcttgggaatcttttcctgtctgtgcctccctgagctgctaaaggtctctggtgtttgtaagaggtggtatcgcctagcgtctgatgagtctctatggcagaccttagacctcacaggtaaaaatctgcacccggatgtgactggtcggttgctgtctcaaggggtgattgccttccgctgcccacgatcatttatggaccaaccattggctgaaggatccgaagttcaactccaagaatcaggcgggggcctggttcaaccaggtggcagtctgaggctgtcatgtacggcctccggcgttacgatttcagcgttgaacgcaatggcgatgggttggtatcgccaagcccctggtgagaggagggtaatggtagctgcggttagtgagcgcgggaacgctatgtatcgagaaagcgttcagggtcgatttacagtgacccgggacttcacaaacaagatggtatctctgcaaatggataatttgaaaccggaggacacggctgtttattattgccacgtccttgaggaccgagtggatagcttccacgattattggggacaggggacgcaagtaacggtcagtagt

SEQ ID NO: 32 - DNA, 927 bp, synthetic construct
  source 1..927: mol_type = other DNA
  misc_feature 1..927: note = nucleotide sequence of Flag tag-E1.GS.NbALFA
gactacaaggacgacgatgacaagacgcgtcgcaggaggcacctccaggagattccaggcctgagtagcaacgttgccaccagcttcacgtggggacgggattccagcaagacttctgaactgctgtcaggcatgggggtctccgccctggagaaagaggagcccgacagtgagaacatcccccaggaactgctctcaaacccgggccacccggagagccccccacggaaacggctgaagagcaaagggagtgacaaagactttgtgattgtccgcaggcctaagctaaaccgagagaactttccaggcgtttcatgggactcccttccggatgagctgctcttgagaatcttttcccgtctgcgcctccctgagctgctaaaggtctctggtgttagtaagaggtggtatcgcctagcgtctgatgagtctctatggaagagcttagacctcacaggtaaaaatctgcacccggatgtgactggtcggttgctgtcccaaggggtggttgccttccgctgcccacgatcatttatggaccaaccattggctggaggatccgaagttcaactccaagaatcaggcgggggcctggttcaaccaggtggcagtctgaggctgtcatgtacggcctccggcgttacgatttcagcgttgaacgcaatggcgatgggttggtatcgccaagcccctggtgagaggagggtaatggtagctgcggttagtgagcgcgggaacgctatgtatcgagaaagcgttcagggtcgatttacagtgacccgggacttcacaaacaagatggtatctctgcaaatggataatttgaaaccggaggacacggctgtttattattgccacgtccttgaggaccgagtggatagcttccacgattattggggacaggggacgcaagtaacggtcagtagt

SEQ ID NO: 33 - DNA, 927 bp, synthetic construct
  source 1..927: mol_type = other DNA
  misc_feature 1..927: note = nucleotide sequence of Flag tag-E2.GS.NbALFA
gactacaaggacgacgatgacaagacgcgtcgcaggaggcacctccaggagattccaggcctgagtagcaacgttgccaccagcttcacgtggggacgggattccagcaagacttctgaactgctgtcaggcatgggggtctccgccctggagaaagaggagcccgacagtgagaacatcccccaggaactgctctcaaacccgggccacccggagagccccccacggaaacggctgaagagcaaagggagtgacaaagactttgtgattgtccgcaggcctaagctaaaccgagagaactttccaggcgtttcatgggactcccttccggatgagctgctcttgagaatcttttcccgtctgcgcctccctgagctgctaaaggtctctggtgttagtaagaggtggtgtcgcctagcgtctgatgagtctctatggaagaccttagacctcacaggtaaaaatctgcacccggatgtgactggtcggttgctgtcccaaggggtggctgccttccgctgcccacgatcatttatggaccaaccattggctggaggatccgaagttcaactccaagaatcaggcgggggcctggttcaaccaggtggcagtctgaggctgtcatgtacggcctccggcgttacgatttcagcgttgaacgcaatggcgatgggttggtatcgccaagcccctggtgagaggagggtaatggtagctgcggttagtgagcgcgggaacgctatgtatcgagaaagcgttcagggtcgatttacagtgacccgggacttcacaaacaagatggtatctctgcaaatggataatttgaaaccggaggacacggctgtttattattgccacgtccttgaggaccgagtggatagcttccacgattattggggacaggggacgcaagtaacggtcagtagt

SEQ ID NO: 34 - DNA, 927 bp, synthetic construct
  source 1..927: mol_type = other DNA
  misc_feature 1..927: note = nucleotide sequence of Flag tag-E4.GS.NbALFA
gactacaaggacgacgatgacaagacgcgtcacaggaagcacctccaggagattccagacccgagtagcaacgttgccaccagcttcacgtggggatgggattccagcaagacttctgaactgccgtcaggcatgggggtctccgccctggagaaagaggagcccgacagtgagaatatcccccaggaactgctctcaaacctgggccacccggagagccccccacggaaacggctgaagagcaaagggagtgacaaaggctttgtgattgtccgcaggcctaagctaaatcgagagaactttccaggtgtttcgtgggtctcccttccggatgagctgctcttgggaatcttttcctgtccgtgcctccctgagctgctaaaggtctctggtgtttgcaagaggtggtgtcgcctagcgtctgatgagcctctatggcagaccttagacctcacaggtaaaaatctgcgcccggatgtgactggtcggttgcggtctcaaggggtgattgccttccgctgccctcggtcatttatggaccaaccattggccgaaggatccgaagttcaactccaagaatcaggcgggggcctggttcaaccaggtggcagtctgaggctgtcatgtacggcctccggcgttacgatttcagcgttgaacgcaatggcgatgggttggtatcgccaagcccctggtgagaggagggtaatggtagctgcggttagtgagcgcgggaacgctatgtatcgagaaagcgttcagggtcgatttacagtgacccgggacttcacaaacaagatggtatctctgcaaatggataatttgaaaccggaggacacggctgtttattattgccacgtccttgaggaccgagtggatagcttccacgattattggggacaggggacgcaagtaacggtcagtagt

SEQ ID NO: 35 - DNA, 927 bp, synthetic construct
  source 1..927: mol_type = other DNA
  misc_feature 1..927: note = nucleotide sequence of Flag tag-E5.GS.NbALFA
gactacaaggacgacgatgacaagacgcgtcacaggaagcacctccaggagattccagacccgagtagcaacgttgccaccagcttcacgtggggatgggattccagcaagacttctgaactgccgtcaggcatgggggtctccgccctggagaaaaaggagcccgacagtgagaatatcccccaggaactgctctcaaacctgggccacccggagagccccccacggaaacggctgaagagcaaagggagtgacaaaggctttgtgattgtccgcaggcctaagctaaatcgtgagaactttccaggtgtttcgtgggtctcccttccggatgagctgctcttgggaatcttttcctgtccgtgcctccctgagctgctaaaggtctctggtgtttgcaagaggtggtgtcgcctagcgtctgatgagcctctaaggcagaccttagacctcacaggtaaaaatctgcgcccggatgtgactggtcggttgctgtctcaaggggtgattgccttccgctgccctcgatcatttatggaccaaccattggccgaaggatccgaagttcaactccaagaatcaggcgggggcctggttcaaccaggtggcagtctgaggctgtcatgtacggcctccggcgttacgatttcagcgttgaacgcaatggcgatgggttggtatcgccaagcccctggtgagaggagggtaatggtagctgcggttagtgagcgcgggaacgctatgtatcgagaaagcgttcagggtcgatttacagtgacccgggacttcacaaacaagatggtatctctgcaaatggataatttgaaaccggaggacacggctgtttattattgccacgtccttgaggaccgagtggatagcttccacgattattggggacaggggacgcaagtaacggtcagtagt

SEQ ID NO: 36 - DNA, 927 bp, synthetic construct
  source 1..927: mol_type = other DNA
  misc_feature 1..927: note = nucleotide sequence of Flag tag-E6.GS.NbALFA
gactacaaggacgacgatgacaagacgcgtcacaggaagcacctccaggagattccagacccgagtagcaacgttgccaccggcttcacgtggggatgggattccagcaaggcttctgaactgccgtcaggcatgggggtctccgccctggagaaagaggagcccgacagtgagaatatcccccaggaactgctctcaaacctgggccacccggagagccccccacggaaacggctgaagagcaaagggagtgacaaaggctttgtgattgtccgcaggcctaagctaaatcgagagaactttccaggtgtttcgtgggtctcccttccgaatgagctgctcttgggaatcttttcctgtcggtgcctccctgagctgctaaaggtctctggtgtttgtaagaggtggtgtcgccaagcgtctgaagagcctctatggcagaccttagacctcacaggtaaaaatctgcgcccggatgtgactggtcggttgcagtctcaaggggtgattgccttccgctgccctcgatcatttatggaccaaccattggctgaaggatccgaagttcaactccaagaatcaggcgggggcctggttcaaccaggtggcagtctgaggctgtcatgtacggcctccggcgttacgatttcagcgttgaacgcaatggcgatgggttggtatcgccaagcccctggtgagaggagggtaatggtagctgcggttagtgagcgcgggaacgctatgtatcgagaaagcgttcagggtcgatttacagtgacccgggacttcacaaacaagatggtatctctgcaaatggataatttgaaaccggaggacacggctgtttattattgccacgtccttgaggaccgagtggatagcttccacgattattggggacaggggacgcaagtaacggtcagtagt

SEQ ID NO: 37 - DNA, 2400 bp, synthetic construct
  source 1..2400: mol_type = other DNA
  misc_feature 1..2400: note = nucleotide sequence of ALFA-Myc tag.STAT3
tcaaggctggaagaagaactgcggagaagactgacagagcctggatcagagcagaaactcatctcagaagaggatctgggtggaggcggtagcgcccaatggaatcagctacagcagcttgacacacggtacctggagcagctccatcagctctacagtgacagcttcccaatggagctgcggcagtttctggccccttggattgagagtcaagattgggcatatgcggccagcaaagaatcacatgccactttggtgtttcataatctcctgggagagattgaccagcagtatagccgcttcctgcaagagtcgaatgttctctatcagcacaatctacgaagaatcaagcagtttcttcagagcaggtatcttgagaagccaatggagattgcccggattgtggcccggtgcctgtgggaagaatcacgccttctacagactgcagccactgcggcccagcaagggggccaggccaaccaccccacagcagccgtggtgacggagaagcagcagatgctggagcagcaccttcaggatgtccggaagagagtgcaggatctagaacagaaaatgaaagtggtagagaatctccaggatgactttgatttcaactataaaaccctcaagagtcaaggagacatgcaagatctgaatggaaacaaccagtcagtgaccaggcagaagatgcagcagctggaacagatgctcactgcgctggaccagatgcggagaagcatcgtgagtgagctggcggggcttttgtcagcgatggagtacgtgcagaaaactctcacggacgaggagctggctgactggaagaggcggcaacagattgcctgcattggaggcccgcccaacatctgcctagatcggctagaaaactggataacgtcattagcagaatctcaacttcagacccgtcaacaaattaagaaactggaggagttgcagcaaaaagtttcctacaaaggggaccccattgtacagcaccggccgatgctggaggagagaatcgtggagctgtttagaaacttaatgaaaagtgcctttgtggtggagcggcagccctgcatgcccatgcatcctgaccggcccctcgtcatcaagaccggcgtccagttcactactaaagtcaggttgctggtcaaattccctgagttgaattatcagcttaaaattaaagtgtgcattgacaaagactctggggacgttgcagctctcagaggatcccggaaatttaacattctgggcacaaacacaaaagtgatgaacatggaagaatccaacaacggcagcctctctgcagaattcaaacacttgaccctgagggagcagagatgtgggaatgggggccgagccaattgtgatgcttccctgattgtgactgaggagctgcacctgatcacctttgagaccgaggtgtatcaccaaggcctcaagattgacctagagacccactccttgccagttgtggtgatctccaacatctgtcagatgccaaatgcctgggcgtccatcctgtggtacaacatgctgaccaacaatcccaagaatgtaaacttttttaccaagcccccaattggaacctgggatcaagtggccgaggtcctgagctggcagttctcctccaccaccaagcgaggactgagcatcgagcagctgactacactggcagagaaactcttgggacctggtgtgaattattcagggtgtcagatcacatgggctaaattttgcaaagaaaacatggctggcaagggcttctccttctgggtctggctggacaatatcattgaccttgtgaaaaagtacatcctggccctttggaacgaagggtacatcatgggctttatcagtaaggagcgggagcgggccatcttgagcactaagcctccaggcaccttcctgctaagattcagtgaaagcagcaaagaaggaggcgtcactttcacttgggtggagaaggacatcagcggtaagacccagatccagtccgtggaaccatacacaaagcagcagctgaacaacatgtcatttgctgaaatcatcatgggctataagatcatggatgctaccaatatcctggtgtctccactggtctatctctatcctgacattcccaaggaggaggcattcggaaagtattgtcggccagagagccaggagcatcctgaagctgacccaggtagcgctgccccatacctgaagaccaagtttatctgtgtgacaccaacgacctgcagcaataccattgacctgccgatgtccccccgcactttagattcattgatgcagtttggaaataatggtgaaggtgctgaaccctcagcaggagggcagtttgagtccctcacctttgacatggagttgacctcggagtgcgctacctcccccatg

SEQ ID NO: 38 - DNA, 2352 bp, synthetic construct
  source 1..2352: mol_type = other DNA
  misc_feature 1..2352: note = nucleotide sequence of Myc tag.STAT3
gagcagaaactcatctcagaagaggatctgggtggaggcggtagcgcccaatggaatcagctacagcagcttgacacacggtacctggagcagctccatcagctctacagtgacagcttcccaatggagctgcggcagtttctggccccttggattgagagtcaagattgggcatatgcggccagcaaagaatcacatgccactttggtgtttcataatctcctgggagagattgaccagcagtatagccgcttcctgcaagagtcgaatgttctctatcagcacaatctacgaagaatcaagcagtttcttcagagcaggtatcttgagaagccaatggagattgcccggattgtggcccggtgcctgtgggaagaatcacgccttctacagactgcagccactgcggcccagcaagggggccaggccaaccaccccacagcagccgtggtgacggagaagcagcagatgctggagcagcaccttcaggatgtccggaagagagtgcaggatctagaacagaaaatgaaagtggtagagaatctccaggatgactttgatttcaactataaaaccctcaagagtcaaggagacatgcaagatctgaatggaaacaaccagtcagtgaccaggcagaagatgcagcagctggaacagatgctcactgcgctggaccagatgcggagaagcatcgtgagtgagctggcggggcttttgtcagcgatggagtacgtgcagaaaactctcacggacgaggagctggctgactggaagaggcggcaacagattgcctgcattggaggcccgcccaacatctgcctagatcggctagaaaactggataacgtcattagcagaatctcaacttcagacccgtcaacaaattaagaaactggaggagttgcagcaaaaagtttcctacaaaggggaccccattgtacagcaccggccgatgctggaggagagaatcgtggagctgtttagaaacttaatgaaaagtgcctttgtggtggagcggcagccctgcatgcccatgcatcctgaccggcccctcgtcatcaagaccggcgtccagttcactactaaagtcaggttgctggtcaaattccctgagttgaattatcagcttaaaattaaagtgtgcattgacaaagactctggggacgttgcagctctcagaggatcccggaaatttaacattctgggcacaaacacaaaagtgatgaacatggaagaatccaacaacggcagcctctctgcagaattcaaacacttgaccctgagggagcagagatgtgggaatgggggccgagccaattgtgatgcttccctgattgtgactgaggagctgcacctgatcacctttgagaccgaggtgtatcaccaaggcctcaagattgacctagagacccactccttgccagttgtggtgatctccaacatctgtcagatgccaaatgcctgggcgtccatcctgtggtacaacatgctgaccaacaatcccaagaatgtaaacttttttaccaagcccccaattggaacctgggatcaagtggccgaggtcctgagctggcagttctcctccaccaccaagcgaggactgagcatcgagcagctgactacactggcagagaaactcttgggacctggtgtgaattattcagggtgtcagatcacatgggctaaattttgcaaagaaaacatggctggcaagggcttctccttctgggtctggctggacaatatcattgaccttgtgaaaaagtacatcctggccctttggaacgaagggtacatcatgggctttatcagtaaggagcgggagcgggccatcttgagcactaagcctccaggcaccttcctgctaagattcagtgaaagcagcaaagaaggaggcgtcactttcacttgggtggagaaggacatcagcggtaagacccagatccagtccgtggaaccatacacaaagcagcagctgaacaacatgtcatttgctgaaatcatcatgggctataagatcatggatgctaccaatatcctggtgtctccactggtctatctctatcctgacattcccaaggaggaggcattcggaaagtattgtcggccagagagccaggagcatcctgaagctgacccaggtagcgctgccccatacctgaagaccaagtttatctgtgtgacaccaacgacctgcagcaataccattgacctgccgatgtccccccgcactttagattcattgatgcagtttggaaataatggtgaaggtgctgaaccctcagcaggagggcagtttgagtccctcacctttgacatggagttgacctcggagtgcgctacctcccccatg

SEQ ID NO: 39 - DNA, 942 bp, synthetic construct
  source 1..942: mol_type = other DNA
  misc_feature 1..942: note = nucleotide sequence of Flag tag-SKP2(2-176).GS.ETI01_A4
gactacaaggacgacgatgacaagacgcgtcacaggaagcacctccaggagattccagacctgagtagcaacgttgccaccagcttcacgtggggatgggattccagcaagacttctgaactgctgtcaggcatgggggtctccgccctggagaaagaggagcccgacagtgagaacatcccccaggaactgctctcaaacctgggccacccggagagccccccacggaaacggctgaagagcaaagggagtgacaaagactttgtgattgtccgcaggcctaagctaaatcgagagaactttccaggtgtttcatgggactcccttccggatgagctgctcttgggaatcttttcctgtctgtgcctccctgagctgctaaaggtctctggtgtttgtaagaggtggtatcgcctagcgtctgatgagtctctatggcagaccttagacctcacaggtaaaaatctgcacccggatgtgactggtcggttgctgtctcaaggggtgattgccttccgctgcccacgatcatttatggaccaaccattggctgaaggatcccatgttcagcttgtagaaagtgggggaggctccgttcaagctggtgggagccttcggctgtcttgtgcagcgagcggttttaactcgggtgatagttgcattggttggttccgacaggttccgggtaaagagcgagagggcgtaagtgtgatttcttccggcggggagattaggtattatgctgatagtgttaagggacgctttacaatctctcaggataataccaaaaacaccctgtatttgcaaatgaactctcttaagcctgaagatacggcaatgtactactgcgccacctccgtttttctgtgttacccgaggacgtggttcaataggtatatgtataactcatggggtcagggaacccaggtaacggtcagtagc

SEQ ID NO: 40 - DNA, 942 bp, synthetic construct
  source 1..942: mol_type = other DNA
  misc_feature 1..942: note = nucleotide sequence of Flag tag-E1.GS.ETI01_A4
gactacaaggacgacgatgacaagacgcgtcgcaggaggcacctccaggagattccaggcctgagtagcaacgttgccaccagcttcacgtggggacgggattccagcaagacttctgaactgctgtcaggcatgggggtctccgccctggagaaagaggagcccgacagtgagaacatcccccaggaactgctctcaaacccgggccacccggagagccccccacggaaacggctgaagagcaaagggagtgacaaagactttgtgattgtccgcaggcctaagctaaaccgagagaactttccaggcgtttcatgggactcccttccggatgagctgctcttgagaatcttttcccgtctgcgcctccctgagctgctaaaggtctctggtgttagtaagaggtggtatcgcctagcgtctgatgagtctctatggaagagcttagacctcacaggtaaaaatctgcacccggatgtgactggtcggttgctgtcccaaggggtggttgccttccgctgcccacgatcatttatggaccaaccattggctggaggatcccatgttcagcttgtagaaagtgggggaggctccgttcaagctggtgggagccttcggctgtcttgtgcagcgagcggttttaactcgggtgatagttgcattggttggttccgacaggttccgggtaaagagcgagagggcgtaagtgtgatttcttccggcggggagattaggtattatgctgatagtgttaagggacgctttacaatctctcaggataataccaaaaacaccctgtatttgcaaatgaactctcttaagcctgaagatacggcaatgtactactgcgccacctccgtttttctgtgttacccgaggacgtggttcaataggtatatgtataactcatggggtcagggaacccaggtaacggtcagtagc

SEQ ID NO: 41 - DNA, 942 bp, synthetic construct
  source 1..942: mol_type = other DNA
  misc_feature 1..942: note = nucleotide sequence of Flag tag-E2.GS.ETI01_A4
gactacaaggacgacgatgacaagacgcgtcgcaggaggcacctccaggagattccaggcctgagtagcaacgttgccaccagcttcacgtggggacgggattccagcaagacttctgaactgctgtcaggcatgggggtctccgccctggagaaagaggagcccgacagtgagaacatcccccaggaactgctctcaaacccgggccacccggagagccccccacggaaacggctgaagagcaaagggagtgacaaagactttgtgattgtccgcaggcctaagctaaaccgagagaactttccaggcgtttcatgggactcccttccggatgagctgctcttgagaatcttttcccgtctgcgcctccctgagctgctaaaggtctctggtgttagtaagaggtggtgtcgcctagcgtctgatgagtctctatggaagaccttagacctcacaggtaaaaatctgcacccggatgtgactggtcggttgctgtcccaaggggtggctgccttccgctgcccacgatcatttatggaccaaccattggctggaggatcccatgttcagcttgtagaaagtgggggaggctccgttcaagctggtgggagccttcggctgtcttgtgcagcgagcggttttaactcgggtgatagttgcattggttggttccgacaggttccgggtaaagagcgagagggcgtaagtgtgatttcttccggcggggagattaggtattatgctgatagtgttaagggacgctttacaatctctcaggataataccaaaaacaccctgtatttgcaaatgaactctcttaagcctgaagatacggcaatgtactactgcgccacctccgtttttctgtgttacccgaggacgtggttcaataggtatatgtataactcatggggtcagggaacccaggtaacggtcagtagc

SEQ ID NO: 42 - DNA, 942 bp, synthetic construct
  source 1..942: mol_type = other DNA
  misc_feature 1..942: note = nucleotide sequence of Flag tag-E4.GS.ETI01_A4
gactacaaggacgacgatgacaagacgcgtcacaggaagcacctccaggagattccagacccgagtagcaacgttgccaccagcttcacgtggggatgggattccagcaagacttctgaactgccgtcaggcatgggggtctccgccctggagaaagaggagcccgacagtgagaatatcccccaggaactgctctcaaacctgggccacccggagagccccccacggaaacggctgaagagcaaagggagtgacaaaggctttgtgattgtccgcaggcctaagctaaatcgagagaactttccaggtgtttcgtgggtctcccttccggatgagctgctcttgggaatcttttcctgtccgtgcctccctgagctgctaaaggtctctggtgtttgcaagaggtggtgtcgcctagcgtctgatgagcctctatggcagaccttagacctcacaggtaaaaatctgcgcccggatgtgactggtcggttgcggtctcaaggggtgattgccttccgctgccctcggtcatttatggaccaaccattggccgaaggatcccatgttcagcttgtagaaagtgggggaggctccgttcaagctggtgggagccttcggctgtcttgtgcagcgagcggttttaactcgggtgatagttgcattggttggttccgacaggttccgggtaaagagcgagagggcgtaagtgtgatttcttccggcggggagattaggtattatgctgatagtgttaagggacgctttacaatctctcaggataataccaaaaacaccctgtatttgcaaatgaactctcttaagcctgaagatacggcaatgtactactgcgccacctccgtttttctgtgttacccgaggacgtggttcaataggtatatgtataactcatggggtcagggaacccaggtaacggtcagtagc

SEQ ID NO: 43 - DNA, 942 bp, synthetic construct
  source 1..942: mol_type = other DNA
  misc_feature 1..942: note = nucleotide sequence of Flag tag-E5.GS.ETI01_A4
gactacaaggacgacgatgacaagacgcgtcacaggaagcacctccaggagattccagacccgagtagcaacgttgccaccagcttcacgtggggatgggattccagcaagacttctgaactgccgtcaggcatgggggtctccgccctggagaaaaaggagcccgacagtgagaatatcccccaggaactgctctcaaacctgggccacccggagagccccccacggaaacggctgaagagcaaagggagtgacaaaggctttgtgattgtccgcaggcctaagctaaatcgtgagaactttccaggtgtttcgtgggtctcccttccggatgagctgctcttgggaatcttttcctgtccgtgcctccctgagctgctaaaggtctctggtgtttgcaagaggtggtgtcgcctagcgtctgatgagcctctaaggcagaccttagacctcacaggtaaaaatctgcgcccggatgtgactggtcggttgctgtctcaaggggtgattgccttccgctgccctcgatcatttatggaccaaccattggccgaaggatcccatgttcagcttgtagaaagtgggggaggctccgttcaagctggtgggagccttcggctgtcttgtgcagcgagcggttttaactcgggtgatagttgcattggttggttccgacaggttccgggtaaagagcgagagggcgtaagtgtgatttcttccggcggggagattaggtattatgctgatagtgttaagggacgctttacaatctctcaggataataccaaaaacaccctgtatttgcaaatgaactctcttaagcctgaagatacggcaatgtactactgcgccacctccgtttttctgtgttacccgaggacgtggttcaataggtatatgtataactcatggggtcagggaacccaggtaacggtcagtagc

SEQ ID NO: 44 - DNA, 942 bp, synthetic construct
  source 1..942: mol_type = other DNA
  misc_feature 1..942: note = nucleotide sequence of Flag tag-E6.GS.ETI01_A4
gactacaaggacgacgatgacaagacgcgtcacaggaagcacctccaggagattccagacccgagtagcaacgttgccaccggcttcacgtggggatgggattccagcaaggcttctgaactgccgtcaggcatgggggtctccgccctggagaaagaggagcccgacagtgagaatatcccccaggaactgctctcaaacctgggccacccggagagccccccacggaaacggctgaagagcaaagggagtgacaaaggctttgtgattgtccgcaggcctaagctaaatcgagagaactttccaggtgtttcgtgggtctcccttccgaatgagctgctcttgggaatcttttcctgtcggtgcctccctgagctgctaaaggtctctggtgtttgtaagaggtggtgtcgccaagcgtctgaagagcctctatggcagaccttagacctcacaggtaaaaatctgcgcccggatgtgactggtcggttgcagtctcaaggggtgattgccttccgctgccctcgatcatttatggaccaaccattggctgaaggatcccatgttcagcttgtagaaagtgggggaggctccgttcaagctggtgggagccttcggctgtcttgtgcagcgagcggttttaactcgggtgatagttgcattggttggttccgacaggttccgggtaaagagcgagagggcgtaagtgtgatttcttccggcggggagattaggtattatgctgatagtgttaagggacgctttacaatctctcaggataataccaaaaacaccctgtatttgcaaatgaactctcttaagcctgaagatacggcaatgtactactgcgccacctccgtttttctgtgttacccgaggacgtggttcaataggtatatgtataactcatggggtcagggaacccaggtaacggtcagtagc

SEQ ID NO: 45 - protein, 122 aa, synthetic construct
  REGION 1..122: note = NbALFA
EVQLQESGGGLVQPGGSLRLSCTASGVTISALNAMAMGWYRQAPGERRVMVAAVSERGNAMYRESVQGRFTVTRDFTNKMVSLQMDNLKPEDTAVYYCHVLEDRVDSFHDYWGQGTQVTVSS

SEQ ID NO: 46 - DNA, 366 bp, synthetic construct
  source 1..366: mol_type = other DNA
  misc_feature 1..366: note = nucleotide sequence of NbALFA
gaagttcaactccaagaatcaggcgggggcctggttcaaccaggtggcagtctgaggctgtcatgtacggcctccggcgttacgatttcagcgttgaacgcaatggcgatgggttggtatcgccaagcccctggtgagaggagggtaatggtagctgcggttagtgagcgcgggaacgctatgtatcgagaaagcgttcagggtcgatttacagtgacccgggacttcacaaacaagatggtatctctgcaaatggataatttgaaaccggaggacacggctgtttattattgccacgtccttgaggaccgagtggatagcttccacgattattggggacaggggacgcaagtaacggtcagtagt

SEQ ID NO: 47 - protein, 424 aa, synthetic construct
  REGION 1..420: note = SKP2 full length
MHRKHLQEIPDLSSNVATSFTWGWDSSKTSELLSGMGVSALEKEEPDSENIPQELLSNLGHPESPPRKRLKSKGSDKDFVIVRRPKLNRENFPGVSWDSLPDELLLGIFSCLCLPELLKVSGVCKRWYRLASDESLWQTLDLTGKNLHPDVTGRLLSQGVIAFRCPRSFMDQPLAEHFSPFRVQHMDLSNSVIEVSTLHGILSQCSKLQNLSLEGLRLSDPIVNTLAKNSNLVRLNLSGCSGFSEFALQTLLSSCSRLDELNLSWCFDFTEKHVQVAVAHVSETITQLNLSGYRKNLQKSDLSTLVRRCPNLVHLDLSDSVMLKNDCFQEFFQLNYLQHLSLSRCYDIIPETLLELGEIPTLKTLQVFGIVPDGTLQLLKEALPHLQINCSHFTTIARPTIGNKKNQEIWGIKCRLTLQKPSCL

SEQ ID NO: 48 - skipped

SEQ ID NO: 49 - protein, 304 aa, synthetic construct
  REGION 1..304: note = SKP2(2-176).GS.ETI01_A4
HRKHLQEIPDLSSNVATSFTWGWDSSKTSELLSGMGVSALEKEEPDSENIPQELLSNLGHPESPPRKRLKSKGSDKDFVIVRRPKLNRENFPGVSWDSLPDELLLGIFSCLCLPELLKVSGVCKRWYRLASDESLWQTLDLTGKNLHPDVTGRLLSQGVIAFRCPRSFMDQPLAEGSHVQLVESGGGSVQAGGSLRLSCAASGFNSGDSCIGWFRQVPGKEREGVSVISSGGEIRYYADSVKGRFTISQDNTKNTLYLQMNSLKPEDTAMYYCATSVFLCYPRTWFNRYMYNSWGQGTQVTVSS

SEQ ID NO: 50 - protein, 7 aa, synthetic construct
  REGION 1..7: note = SKP2(2-176)V3.GS.ETI01_A4
AAAAAAA

SEQ ID NO: 51 - protein, 7 aa, synthetic construct
  REGION 1..7: note = SKP2(2-176)V15.GS.ETI01_A4
AAAAAAA

SEQ ID NO: 52 - protein, 304 aa, synthetic construct
  REGION 1..304: note = E1.GS.ETI01_A4
RRRHLQEIPGLSSNVATSFTWGRDSSKTSELLSGMGVSALEKEEPDSENIPQELLSNPGHPESPPRKRLKSKGSDKDFVIVRRPKLNRENFPGVSWDSLPDELLLRIFSRLRLPELLKVSGVSKRWYRLASDESLWKSLDLTGKNLHPDVTGRLLSQGVVAFRCPRSFMDQPLAGGSHVQLVESGGGSVQAGGSLRLSCAASGFNSGDSCIGWFRQVPGKEREGVSVISSGGEIRYYADSVKGRFTISQDNTKNTLYLQMNSLKPEDTAMYYCATSVFLCYPRTWFNRYMYNSWGQGTQVTVSS

SEQ ID NO: 53 - protein, 304 aa, synthetic construct
  REGION 1..304: note = E2.GS.ETI01_A4
RRRHLQEIPGLSSNVATSFTWGRDSSKTSELLSGMGVSALEKEEPDSENIPQELLSNPGHPESPPRKRLKSKGSDKDFVIVRRPKLNRENFPGVSWDSLPDELLLRIFSRLRLPELLKVSGVSKRWCRLASDESLWKTLDLTGKNLHPDVTGRLLSQGVAAFRCPRSFMDQPLAGGSHVQLVESGGGSVQAGGSLRLSCAASGFNSGDSCIGWFRQVPGKEREGVSVISSGGEIRYYADSVKGRFTISQDNTKNTLYLQMNSLKPEDTAMYYCATSVFLCYPRTWFNRYMYNSWGQGTQVTVSS

SEQ ID NO: 54 - protein, 304 aa, synthetic construct
  REGION 1..304: note = E4.GS.ETI01_A4
HRKHLQEIPDPSSNVATSFTWGWDSSKTSELPSGMGVSALEKEEPDSENIPQELLSNLGHPESPPRKRLKSKGSDKGFVIVRRPKLNRENFPGVSWVSLPDELLLGIFSCPCLPELLKVSGVCKRWCRLASDEPLWQTLDLTGKNLRPDVTGRLRSQGVIAFRCPRSFMDQPLAEGSHVQLVESGGGSVQAGGSLRLSCAASGFNSGDSCIGWFRQVPGKEREGVSVISSGGEIRYYADSVKGRFTISQDNTKNTLYLQMNSLKPEDTAMYYCATSVFLCYPRTWFNRYMYNSWGQGTQVTVSS

SEQ ID NO: 55 - protein, 304 aa, synthetic construct
  REGION 1..304: note = E5.GS.ETI01_A4
HRKHLQEIPDPSSNVATSFTWGWDSSKTSELPSGMGVSALEKKEPDSENIPQELLSNLGHPESPPRKRLKSKGSDKGFVIVRRPKLNRENFPGVSWVSLPDELLLGIFSCPCLPELLKVSGVCKRWCRLASDEPLRQTLDLTGKNLRPDVTGRLLSQGVIAFRCPRSFMDQPLAEGSHVQLVESGGGSVQAGGSLRLSCAASGFNSGDSCIGWFRQVPGKEREGVSVISSGGEIRYYADSVKGRFTISQDNTKNTLYLQMNSLKPEDTAMYYCATSVFLCYPRTWFNRYMYNSWGQGTQVTVSS

SEQ ID NO: 56 - protein, 6 aa, synthetic construct
  REGION 1..6: note = E6.GS.ETI01_A4
AAAAAA

SEQ ID NO: 57 - DNA, 912 bp, synthetic construct
  source 1..912: mol_type = other DNA
  misc_feature 1..912: note = SKP2(2-176).GS.ETI01_A4
cacaggaagcacctccaggagattccagacctgagtagcaacgttgccaccagcttcacgtggggatgggattccagcaagacttctgaactgctgtcaggcatgggggtctccgccctggagaaagaggagcccgacagtgagaacatcccccaggaactgctctcaaacctgggccacccggagagccccccacggaaacggctgaagagcaaagggagtgacaaagactttgtgattgtccgcaggcctaagctaaatcgagagaactttccaggtgtttcatgggactcccttccggatgagctgctcttgggaatcttttcctgtctgtgcctccctgagctgctaaaggtctctggtgtttgtaagaggtggtatcgcctagcgtctgatgagtctctatggcagaccttagacctcacaggtaaaaatctgcacccggatgtgactggtcggttgctgtctcaaggggtgattgccttccgctgcccacgatcatttatggaccaaccattggctgaaggatcccatgttcagcttgtagaaagtgggggaggctccgttcaagctggtgggagccttcggctgtcttgtgcagcgagcggttttaactcgggtgatagttgcattggttggttccgacaggttccgggtaaagagcgagagggcgtaagtgtgatttcttccggcggggagattaggtattatgctgatagtgttaagggacgctttacaatctctcaggataataccaaaaacaccctgtatttgcaaatgaactctcttaagcctgaagatacggcaatgtactactgcgccacctccgtttttctgtgttacccgaggacgtggttcaataggtatatgtataactcatggggtcagggaacccaggtaacggtcagtagc

SEQ ID NO: 58 - DNA, 15 bp, synthetic construct
  source 1..15: mol_type = other DNA
  misc_feature 1..15: note = SKP2(2-176)V3.GS.ETI01_A4
aaaaaaaaaaaaaaa

SEQ ID NO: 59 - DNA, 12 bp, synthetic construct
  source 1..12: mol_type = other DNA
  misc_feature 1..11: note = SKP2(2-176)V15.GS.ETI01_A4
aaaaaaaaaaaa

SEQ ID NO: 60 - DNA, 912 bp, synthetic construct
  source 1..912: mol_type = other DNA
  misc_feature 1..912: note = E1.GS.ETI01_A4
cgcaggaggcacctccaggagattccaggcctgagtagcaacgttgccaccagcttcacgtggggacgggattccagcaagacttctgaactgctgtcaggcatgggggtctccgccctggagaaagaggagcccgacagtgagaacatcccccaggaactgctctcaaacccgggccacccggagagccccccacggaaacggctgaagagcaaagggagtgacaaagactttgtgattgtccgcaggcctaagctaaaccgagagaactttccaggcgtttcatgggactcccttccggatgagctgctcttgagaatcttttcccgtctgcgcctccctgagctgctaaaggtctctggtgttagtaagaggtggtatcgcctagcgtctgatgagtctctatggaagagcttagacctcacaggtaaaaatctgcacccggatgtgactggtcggttgctgtcccaaggggtggttgccttccgctgcccacgatcatttatggaccaaccattggctggaggatcccatgttcagcttgtagaaagtgggggaggctccgttcaagctggtgggagccttcggctgtcttgtgcagcgagcggttttaactcgggtgatagttgcattggttggttccgacaggttccgggtaaagagcgagagggcgtaagtgtgatttcttccggcggggagattaggtattatgctgatagtgttaagggacgctttacaatctctcaggataataccaaaaacaccctgtatttgcaaatgaactctcttaagcctgaagatacggcaatgtactactgcgccacctccgtttttctgtgttacccgaggacgtggttcaataggtatatgtataactcatggggtcagggaacccaggtaacggtcagtagc

SEQ ID NO: 61 - DNA, 912 bp, synthetic construct
  source 1..912: mol_type = other DNA
  misc_feature 1..912: note = E2.GS.ETI01_A4
cgcaggaggcacctccaggagattccaggcctgagtagcaacgttgccaccagcttcacgtggggacgggattccagcaagacttctgaactgctgtcaggcatgggggtctccgccctggagaaagaggagcccgacagtgagaacatcccccaggaactgctctcaaacccgggccacccggagagccccccacggaaacggctgaagagcaaagggagtgacaaagactttgtgattgtccgcaggcctaagctaaaccgagagaactttccaggcgtttcatgggactcccttccggatgagctgctcttgagaatcttttcccgtctgcgcctccctgagctgctaaaggtctctggtgttagtaagaggtggtgtcgcctagcgtctgatgagtctctatggaagaccttagacctcacaggtaaaaatctgcacccggatgtgactggtcggttgctgtcccaaggggtggctgccttccgctgcccacgatcatttatggaccaaccattggctggaggatcccatgttcagcttgtagaaagtgggggaggctccgttcaagctggtgggagccttcggctgtcttgtgcagcgagcggttttaactcgggtgatagttgcattggttggttccgacaggttccgggtaaagagcgagagggcgtaagtgtgatttcttccggcggggagattaggtattatgctgatagtgttaagggacgctttacaatctctcaggataataccaaaaacaccctgtatttgcaaatgaactctcttaagcctgaagatacggcaatgtactactgcgccacctccgtttttctgtgttacccgaggacgtggttcaataggtatatgtataactcatggggtcagggaacccaggtaacggtcagtagc

SEQ ID NO: 62 - DNA, 912 bp, synthetic construct
  source 1..912: mol_type = other DNA
  misc_feature 1..912: note = E4.GS.ETI01_A4
cacaggaagcacctccaggagattccagacccgagtagcaacgttgccaccagcttcacgtggggatgggattccagcaagacttctgaactgccgtcaggcatgggggtctccgccctggagaaagaggagcccgacagtgagaatatcccccaggaactgctctcaaacctgggccacccggagagccccccacggaaacggctgaagagcaaagggagtgacaaaggctttgtgattgtccgcaggcctaagctaaatcgagagaactttccaggtgtttcgtgggtctcccttccggatgagctgctcttgggaatcttttcctgtccgtgcctccctgagctgctaaaggtctctggtgtttgcaagaggtggtgtcgcctagcgtctgatgagcctctatggcagaccttagacctcacaggtaaaaatctgcgcccggatgtgactggtcggttgcggtctcaaggggtgattgccttccgctgccctcggtcatttatggaccaaccattggccgaaggatcccatgttcagcttgtagaaagtgggggaggctccgttcaagctggtgggagccttcggctgtcttgtgcagcgagcggttttaactcgggtgatagttgcattggttggttccgacaggttccgggtaaagagcgagagggcgtaagtgtgatttcttccggcggggagattaggtattatgctgatagtgttaagggacgctttacaatctctcaggataataccaaaaacaccctgtatttgcaaatgaactctcttaagcctgaagatacggcaatgtactactgcgccacctccgtttttctgtgttacccgaggacgtggttcaataggtatatgtataactcatggggtcagggaacccaggtaacggtcagtagc

SEQ ID NO: 63 - DNA, 912 bp, synthetic construct
  source 1..912: mol_type = other DNA
  misc_feature 1..912: note = E5.GS.ETI01_A4
cacaggaagcacctccaggagattccagacccgagtagcaacgttgccaccagcttcacgtggggatgggattccagcaagacttctgaactgccgtcaggcatgggggtctccgccctggagaaaaaggagcccgacagtgagaatatcccccaggaactgctctcaaacctgggccacccggagagccccccacggaaacggctgaagagcaaagggagtgacaaaggctttgtgattgtccgcaggcctaagctaaatcgtgagaactttccaggtgtttcgtgggtctcccttccggatgagctgctcttgggaatcttttcctgtccgtgcctccctgagctgctaaaggtctctggtgtttgcaagaggtggtgtcgcctagcgtctgatgagcctctaaggcagaccttagacctcacaggtaaaaatctgcgcccggatgtgactggtcggttgctgtctcaaggggtgattgccttccgctgccctcgatcatttatggaccaaccattggccgaaggatcccatgttcagcttgtagaaagtgggggaggctccgttcaagctggtgggagccttcggctgtcttgtgcagcgagcggttttaactcgggtgatagttgcattggttggttccgacaggttccgggtaaagagcgagagggcgtaagtgtgatttcttccggcggggagattaggtattatgctgatagtgttaagggacgctttacaatctctcaggataataccaaaaacaccctgtatttgcaaatgaactctcttaagcctgaagatacggcaatgtactactgcgccacctccgtttttctgtgttacccgaggacgtggttcaataggtatatgtataactcatggggtcagggaacccaggtaacggtcagtagc

SEQ ID NO: 64 - DNA, 12 bp, synthetic construct
  source 1..12: mol_type = other DNA
  misc_feature 1..12: note = E6.GS.ETI01_A4
aaaaaaaaaaaa

SEQ ID NO: 65 - protein, 127 aa, synthetic construct
  REGION 1..127: note = ETI01_A4
HVQLVESGGGSVQAGGSLRLSCAASGFNSGDSCIGWFRQVPGKEREGVSVISSGGEIRYYADSVKGRFTISQDNTKNTLYLQMNSLKPEDTAMYYCATSVFLCYPRTWFNRYMYNSWGQGTQVTVSS

SEQ ID NO: 66 - DNA, 381 bp, synthetic construct
  source 1..381: mol_type = other DNA
  misc_feature 1..381: note = nucleotide seqeune coding ETI01_A4
catgttcagcttgtagaaagtgggggaggctccgttcaagctggtgggagccttcggctgtcttgtgcagcgagcggttttaactcgggtgatagttgcattggttggttccgacaggttccgggtaaagagcgagagggcgtaagtgtgatttcttccggcggggagattaggtattatgctgatagtgttaagggacgctttacaatctctcaggataataccaaaaacaccctgtatttgcaaatgaactctcttaagcctgaagatacggcaatgtactactgcgccacctccgtttttctgtgttacccgaggacgtggttcaataggtatatgtataactcatggggtcagggaacccaggtaacggtcagtagc